European Patent Specification EP 3 653 730 B1, published August 16, 2023. Title: Kit for isolation of mutant cell free DNA and method for isolation of mutant cell free DNA using the same. Applicant: GENECKER. The sequence listing filed with the application follows.

SEQUENCE LISTING (19 sequences)

SEQ ID NO: 1 - protein, 1383 aa, Artificial Sequence
  spCas9 with 6His
MGHHHHHHAELPGIRPDKKYSIGLDIGTNSVGWAVITDEYKVPSKKFKVLGNTDRHSIKKNLIGALLFDSGETAEATRLKRTARRRYTRRKNRICYLQEIFSNEMAKVDDSFFHRLEESFLVEEDKKHERHPIFGNIVDEVAYHEKYPTIYHLRKKLVDSTDKADLRLIYLALAHMIKFRGHFLIEGDLNPDNSDVDKLFIQLVQTYNQLFEENPINASGVDAKAILSARLSKSRRLENLIAQLPGEKKNGLFGNLIALSLGLTPNFKSNFDLAEDAKLQLSKDTYDDDLDNLLAQIGDQYADLFLAAKNLSDAILLSDILRVNTEITKAPLSASMIKRYDEHHQDLTLLKALVRQQLPEKYKEIFFDQSKNGYAGYIDGGASQEEFYKFIKPILEKMDGTEELLVKLNREDLLRKQRTFDNGSIPHQIHLGELHAILRRQEDFYPFLKDNREKIEKILTFRIPYYVGPLARGNSRFAWMTRKSEETITPWNFEEVVDKGASAQSFIERMTNFDKNLPNEKVLPKHSLLYEYFTVYNELTKVKYVTEGMRKPAFLSGEQKKAIVDLLFKTNRKVTVKQLKEDYFKKIECFDSVEISGVEDRFNASLGTYHDLLKIIKDKDFLDNEENEDILEDIVLTLTLFEDREMIEERLKTYAHLFDDKVMKQLKRRRYTGWGRLSRKLINGIRDKQSGKTILDFLKSDGFANRNFMQLIHDDSLTFKEDIQKAQVSGQGDSLHEHIANLAGSPAIKKGILQTVKVVDELVKVMGRHKPENIVIEMARENQTTQKGQKNSRERMKRIEEGIKELGSQILKEHPVENTQLQNEKLYLYYLQNGRDMYVDQELDINRLSDYDVDHIVPQSFLKDDSIDNKVLTRSDKNRGKSDNVPSEEVVKKMKNYWRQLLNAKLITQRKFDNLTKAERGGLSELDKAGFIKRQLVETRQITKHVAQILDSRMNTKYDENDKLIREVKVITLKSKLVSDFRKDFQFYKVREINNYHHAHDAYLNAVVGTALIKKYPKLESEFVYGDYKVYDVRKMIAKSEQEIGKATAKYFFYSNIMNFFKTEITLANGEIRKRPLIETNGETGEIVWDKGRDFATVRKVLSMPQVNIVKKTEVQTGGFSKESILPKRNSDKLIARKKDWDPKKYGGFDSPTVAYSVLVVAKVEKGKSKKLKSVKELLGITIMERSSFEKNPIDFLEAKGYKEVKKDLIIKLPKYSLFELENGRKRMLASAGELQKGNELALPSKYVNFLYLASHYEKLKGSPEDNEQKQLFVEQHKHYLDEIIEQISEFSKRVILADANLDKVLSAYNKHRDKPIREQAENIIHLFTLTNLGAPAAFKYFDTTIDRKRYTSTKEVLDATLIHQSITGLYETRIDLSQLGGD

SEQ ID NO: 2 - RNA, 96 nt, Artificial Sequence
  KRAS G12V site targeting sgRNA
aaacuugugguaguuggagcguuuuagagcuagaaauagcaaguuaaaauaaggcuaguccguuaucaacuugaaaaaguggcaccgagucggugc

SEQ ID NO: 3 - RNA, 96 nt, Artificial Sequence
  EGFR Del746-750 site targeting sgRNA
ucuuaauuccuugauagcgaguuuuagagcuagaaauagcaaguuaaaauaaggcuaguccguuaucaacuugaaaaaguggcaccgagucggugc

SEQ ID NO: 4 - DNA, 2786 bp, Homo sapiens
  gene (1)..(2786): KRAS wt target, human
tttgtttgttttgagatggagtcttactccgtcacccaatctggagtgcagtggcgtgatctgggctcactgcaacctctgcctcccgggttcaagtgattctccttcctcagcctccccagtagctaggactacaggagagcgccaccacgcctgattaatttttgtatttttagtagagagagggtttcaccatattggccaggctggtcttgaactcctggcctcaggtgatccacccgccttggcctctgaaagtgctgggattacaggcatgagccgccgcacccggctttctaatctttatctttttttgtgcagcggtgatacaggattatgtattgtactgaacagttaattcggagttctcttggtttttagctttattttccccagagatttttttttttttttttttttttgagacggagtcttgctctatcgccaggctggagtgcagtggcgccatctcggctcattgcaacctcggactcctattttccccagagatatttcacacattaaaatgtcgtcaaatattgttcttctttgcctcagtgtttaaatttttatttccccatgacacaatccagctttatttgacactcattctctcaactctcatctgattcttactgttaatatttatccaagagaactactgccatgatgctttaaaagtttttctgtagctgttgcatattgacttctaacacttagaggtgggggtccactaggaaaactgtaacaataagagtggagatagctgtcagcaacttttgtgagggtgtgctacagggtgtagagcactgtgaagtctctacatgagtgaagtcatgatatgatcctttgagagcctttagccgccgcagaacagcagtctggctatttagatagaacaacttgattttaagataaaagaactgtctatgtagcatttatgcatttttcttaagcgtcgatggaggagtttgtaaatgaagtacagttcattacgatacacgtctgcagtcaactggaattttcatgattgaattttgtaaggtattttgaaataatttttcatataaaggtgagtttgtattaaaaggtactggtggagtatttgatagtgtattaaccttatgtgtgacatgttctaatatagtcacattttcattatttttattataaggcctgctgaaaatgactgaatataaacttgtggtagttggagctggtggcgtaggcaagagtgccttgacgatacagctaattcagaatcattttgtggacgaatatgatccaacaatagaggtaaatcttgttttaatatgcatattactggtgcaggaccattctttgatacagataaaggtttctctgaccattttcatgagtacttattacaagataattatgctgaaagttaagttatctgaaatgtaccttgggtttcaagttatatgtaaccattaatatgggaactttactttccttgggagtatgtcagggtccatgatgttcactctctgtgcattttgattggaagtgtatttcagagtttcgtgagagggtagaaatttgtatcctatctggacctaaaagacaatctttttattgtaacttttatttttatgggtttcttggtattgtgacatcatatgtaaaggttagatttaattgtactagtgaaatataattgtttgatggttgatttttttaaacttcatcagcagtattttcctatcttcttctcaacattagagaacctacaactaccggataaattttacaaaatgaattatttgcctaaggtgtggtttatataaaggtactattaccaactttacctttgctttgttgtcatttttaaatttactcaaggaaatactaggatttaaaaaaaaattccttgagtaaatttaaattgttatcatgtttttgaggattattttcagatttttttagtttaatgaaaatttaccaaagtaaagaccagcagcagaatgataagtaaagacctgtaagacaccttgaaggtcatggagtagaacttccatcccaagcagatgaggatttatttaatctcaaagacctccaggaggggacattccccaactgtccttgttaactcattttcagaacatatttattagcatattttacatgtaatttggatcttcatgttaaatttaacatcagtggagatggaaaataagcatatcgccttgtctttgaaatagccctatattgttagattgtttcttaggcttctttaccctgggttaagcagtcctaatactttagcatttattctacatctagtgtactaatttaaaaaaatcagttctgaaaaatttctaagaactttcttcaagttccaagctgtgaaatctagaacaggtcaaagtgccttattaacgtactgtactgtgtagtgtcttgaagagacactttgcgctgaggcaagttctgagggcattgggtggccttgggaagatatttatgcagtttagaacctggagaattgattagataactaatcataaggaaacgtcacatatttttggtactataaaaaagtggagaaataatgcctatttgcaaagatttgatttaaacatagaaacaactttatttggcttccaattttaagaatttacagcagtaaaggggaacagtctaattgaagtagactgcctatgcaatagtctctgtatatttacttttgacaagttaattcaatgtgtactatagttttgtttctttgaagaggtttgaatagtgcacccattttaatctgt

SEQ ID NO: 5 - protein, 186 aa, Homo sapiens
  PEPTIDE (1)..(186): wt KRAS Amino Acids
MTEYKLVVVGAGGVGKSALTIQLIQNHFVDEYDPTIEDSYRKQVVIDGETCLLDILDTAGQEEYSAMRDQYMRTGEGFLCVFAINNTKSFEDIHHYREQIKRVKDSEDVPMVLVGNKCDLPSRTVDTKQAQDLARSYGIPFIETSAKTRQRVEDAFYTLVREIRQYRLKKISKEEKTPGCVKIKKC

SEQ ID NO: 6 - DNA, 2787 bp, Homo sapiens
  gene (1)..(2787): KRAS MUTANT G12V target , HUMAN
gtttgtttgttttgagatggagtcttactccgtcacccaatctggagtgcagtggcgtgatctgggctcactgcaacctctgcctcccgggttcaagtgattctccttcctcagcctccccagtagctaggactacaggagagcgccaccacgcctgattaatttttgtatttttagtagagagagggtttcaccatattggccaggctggtcttgaactcctggcctcaggtgatccacccgccttggcctctgaaagtgctgggattacaggcatgagccgccgcacccggctttctaatctttatctttttttgtgcagcggtgatacaggattatgtattgtactgaacagttaattcggagttctcttggtttttagctttattttccccagagatttttttttttttttttttttttgagacggagtcttgctctatcgccaggctggagtgcagtggcgccatctcggctcattgcaacctcggactcctattttccccagagatatttcacacattaaaatgtcgtcaaatattgttcttctttgcctcagtgtttaaatttttatttccccatgacacaatccagctttatttgacactcattctctcaactctcatctgattcttactgttaatatttatccaagagaactactgccatgatgctttaaaagtttttctgtagctgttgcatattgacttctaacacttagaggtgggggtccactaggaaaactgtaacaataagagtggagatagctgtcagcaacttttgtgagggtgtgctacagggtgtagagcactgtgaagtctctacatgagtgaagtcatgatatgatcctttgagagcctttagccgccgcagaacagcagtctggctatttagatagaacaacttgattttaagataaaagaactgtctatgtagcatttatgcatttttcttaagcgtcgatggaggagtttgtaaatgaagtacagttcattacgatacacgtctgcagtcaactggaattttcatgattgaattttgtaaggtattttgaaataatttttcatataaaggtgagtttgtattaaaaggtactggtggagtatttgatagtgtattaaccttatgtgtgacatgttctaatatagtcacattttcattatttttattataaggcctgctgaaaatgactgaatataaacttgtggtagttggagctgttggcgtaggcaagagtgccttgacgatacagctaattcagaatcattttgtggacgaatatgatccaacaatagaggtaaatcttgttttaatatgcatattactggtgcaggaccattctttgatacagataaaggtttctctgaccattttcatgagtacttattacaagataattatgctgaaagttaagttatctgaaatgtaccttgggtttcaagttatatgtaaccattaatatgggaactttactttccttgggagtatgtcagggtccatgatgttcactctctgtgcattttgattggaagtgtatttcagagtttcgtgagagggtagaaatttgtatcctatctggacctaaaagacaatctttttattgtaacttttatttttatgggtttcttggtattgtgacatcatatgtaaaggttagatttaattgtactagtgaaatataattgtttgatggttgatttttttaaacttcatcagcagtattttcctatcttcttctcaacattagagaacctacaactaccggataaattttacaaaatgaattatttgcctaaggtgtggtttatataaaggtactattaccaactttacctttgctttgttgtcatttttaaatttactcaaggaaatactaggatttaaaaaaaaattccttgagtaaatttaaattgttatcatgtttttgaggattattttcagatttttttagtttaatgaaaatttaccaaagtaaagaccagcagcagaatgataagtaaagacctgtaagacaccttgaaggtcatggagtagaacttccatcccaagcagatgaggatttatttaatctcaaagacctccaggaggggacattccccaactgtccttgttaactcattttcagaacatatttattagcatattttacatgtaatttggatcttcatgttaaatttaacatcagtggagatggaaaataagcatatcgccttgtctttgaaatagccctatattgttagattgtttcttaggcttctttaccctgggttaagcagtcctaatactttagcatttattctacatctagtgtactaatttaaaaaaatcagttctgaaaaatttctaagaactttcttcaagttccaagctgtgaaatctagaacaggtcaaagtgccttattaacgtactgtactgtgtagtgtcttgaagagacactttgcgctgaggcaagttctgagggcattgggtggccttgggaagatatttatgcagtttagaacctggagaattgattagataactaatcataaggaaacgtcacatatttttggtactataaaaaagtggagaaataatgcctatttgcaaagatttgatttaaacatagaaacaactttatttggcttccaattttaagaatttacagcagtaaaggggaacagtctaattgaagtagactgcctatgcaatagtctctgtatatttacttttgacaagttaattcaatgtgtactatagttttgtttctttgaagaggtttgaatagtgcacccattttaatctgt

SEQ ID NO: 7 - protein, 186 aa, Homo sapiens
  PEPTIDE (1)..(186): mutant KRAS Amino Acids
MTEYKLVVVGAVGVGKSALTIQLIQNHFVDEYDPTIEDSYRKQVVIDGETCLLDILDTAGQEEYSAMRDQYMRTGEGFLCVFAINNTKSFEDIHHYREQIKRVKDSEDVPMVLVGNKCDLPSRTVDTKQAQDLARSYGIPFIETSAKTRQRVEDAFYTLVREIRQYRLKKISKEEKTPGCVKIKKC

SEQ ID NO: 8 - DNA, 23 bp, Artificial Sequence
  KRAS target site including PAM
aaacttgtggtagttggagctgg

SEQ ID NO: 9 - DNA, 2813 bp, Homo sapiens
  gene (1)..(2813): EGFR wt target sequence, human
ctcataagcataagcgcgtgtgatgtgccccaaccaaacgaccgccatgcacaacttccctaccggagttttcaatccagttaataggcgtggaaacagacatagaaattgtgtttgttgaaaggtagctgttcagttaaagaacacctgtatcagagcctgtgtttctaccaacttctgtcaagctctgtagagaaggcgtacatttgtccttccaaatgagctggcaagtgccgtgtcctggcacccaagcccatgccgtggctgctggtccccctgctgggccatgtctggcactgctttccagcatggtgagggctgaggtgacccttgtctctgtgttcttgtcccccccagcttgtggagcctcttacacccagtggagaagctcccaaccaagctctcttgaggatcttgaaggaaactgaattcaaaaagatcaaagtgctgggctccggtgcgttcggcacggtgtataaggtaaggtccctggcacaggcctctgggctgggccgcagggcctctcatggtctggtggggagcccagagtccttgcaagctgtatatttccatcatctactttactctttgtttcactgagtgtttgggaaactccagtgtttttcccaagttattgagaggaaatcttttataaccacagtaatcagtggtcctgtgagaccaattcacagaccaaaggcatttttatgaaaggggccattgaccttgccatggggtgcagcacagggcgggaggagggccgcctctcaccgcacggcatcagaatgcagcccagctgaaatgggctcatcttcgtttgcttcttctagatcctctttgcatgaaatctgatttcagttaggcctagacgcagcatcattaaattctggatgaaatgatccacacggactttataacaggctttacaagcttgagattcttttatctaaataatcagtgtgattcgtggagcccaacagctgcagggctgcgggggcgtcacagcccccagcaatatcagccttaggtgcggctccacagccccagtgtccctcaccttcggggtgcatcgctggtaacatccacccagatcactgggcagcatgtggcaccatctcacaattgccagttaacgtcttccttctctctctgtcatagggactctggatcccagaaggtgagaaagttaaaattcccgtcgctatcaaggaattaagagaagcaacatctccgaaagccaacaaggaaatcctcgatgtgagtttctgctttgctgtgtgggggtccatggctctgaacctcaggcccaccttttctcatgtctggcagctgctctgctctagaccctgctcatctccacatcctaaatgttcactttctatgtctttccctttctagctctagtgggtataactccctccccttagagacagcactggcctctcccatgctggtatccaccccaaaaggctggaaacaggcaattactggcatctacccagcactagtttcttgacacgcatgatgagtgagtgctcttggtgagcctggagcatgggtattgtttttggtattttttggatgaagaaatggaggcataaagaaattggctgacccttatatggctgggatagggtttaagccccttgttatttctgactctgaaacttgcattcaattcactccaccaagttatctcatctttgaaatggctttttttaaaggtgcctagaatatgatggcgtgcagtctataaactgttgcccaccttctgtactttctctcagaataattcacattcttctccagtgtctgttgattgttactttgtggaataagttcttggaaaattccacaagattattgttatcttcttactaccaattctattgaactttctccaccttctctgggccttccccagccagtggtgggaagatgctggctggagtctgacagagcctcttctacactggcctgggcttgctgtgagttggtggaaacctttgctcttgtcccaacacagagcaagtgaaagaggaggtcaaggggctcaggcagcggactagggaagcagaatcgaggaaaaggaaaaatggctgacttattacctcaaaactctagagaatttagttgatcttacagccaagaaggacaaaagccagagagtaatatcctccgcctcatgtctaacccacagaatacatagcaagtaaagagaacatgggcctttataaaaatgtcttaagatacaattttttaattggaggaaatctacagtttaattttctctgggcagcttttcttccttttattatagtaggggaaatcccatgttgatatacttctaaatgaaagatgatgaattgatataatacaataaaaaatctgtaaaattgatgatatacttatcaagaaaaattagctttcattttaacggtttacaaattgagtcaagtcctagtaacaaaatgttaagtctattaacataaccacaagaaatacaggaagacgggcaatctgtgaagcctttcacttacaatctctggcccctcacctgtgctgtgtaggaaaatctttgtgcacaatttgcttccttaattcattttttattcattcaacacattctaataaattatacaaaatcatgttgaaatgtgaatttcagtggtatttataaatgcagtgtgaggagggtttggatgtattctaagacaatagttgtgctttgggaaggaagcagtgttcactgaaaagtgcccccaggaccttttaattggaggaaatatgcttctgtggagttggaaatgggg

SEQ ID NO: 10 - protein, 1210 aa, Homo sapiens [sequence omitted]

SEQ ID NO: 11 - DNA, 2798 bp, Homo sapiens
  gene (1)..(2798): EGFR Deletion mutant. 746-750
ctcataagcataagcgcgtgtgatgtgccccaaccaaacgaccgccatgcacaacttccctaccggagttttcaatccagttaataggcgtggaaacagacatagaaattgtgtttgttgaaaggtagctgttcagttaaagaacacctgtatcagagcctgtgtttctaccaacttctgtcaagctctgtagagaaggcgtacatttgtccttccaaatgagctggcaagtgccgtgtcctggcacccaagcccatgccgtggctgctggtccccctgctgggccatgtctggcactgctttccagcatggtgagggctgaggtgacccttgtctctgtgttcttgtcccccccagcttgtggagcctcttacacccagtggagaagctcccaaccaagctctcttgaggatcttgaaggaaactgaattcaaaaagatcaaagtgctgggctccggtgcgttcggcacggtgtataaggtaaggtccctggcacaggcctctgggctgggccgcagggcctctcatggtctggtggggagcccagagtccttgcaagctgtatatttccatcatctactttactctttgtttcactgagtgtttgggaaactccagtgtttttcccaagttattgagaggaaatcttttataaccacagtaatcagtggtcctgtgagaccaattcacagaccaaaggcatttttatgaaaggggccattgaccttgccatggggtgcagcacagggcgggaggagggccgcctctcaccgcacggcatcagaatgcagcccagctgaaatgggctcatcttcgtttgcttcttctagatcctctttgcatgaaatctgatttcagttaggcctagacgcagcatcattaaattctggatgaaatgatccacacggactttataacaggctttacaagcttgagattcttttatctaaataatcagtgtgattcgtggagcccaacagctgcagggctgcgggggcgtcacagcccccagcaatatcagccttaggtgcggctccacagccccagtgtccctcaccttcggggtgcatcgctggtaacatccacccagatcactgggcagcatgtggcaccatctcacaattgccagttaacgtcttccttctctctctgtcatagggactctggatcccagaaggtgagaaagttaaaattcccgtcgctatcaagacatctccgaaagccaacaaggaaatcctcgatgtgagtttctgctttgctgtgtgggggtccatggctctgaacctcaggcccaccttttctcatgtctggcagctgctctgctctagaccctgctcatctccacatcctaaatgttcactttctatgtctttccctttctagctctagtgggtataactccctccccttagagacagcactggcctctcccatgctggtatccaccccaaaaggctggaaacaggcaattactggcatctacccagcactagtttcttgacacgcatgatgagtgagtgctcttggtgagcctggagcatgggtattgtttttggtattttttggatgaagaaatggaggcataaagaaattggctgacccttatatggctgggatagggtttaagccccttgttatttctgactctgaaacttgcattcaattcactccaccaagttatctcatctttgaaatggctttttttaaaggtgcctagaatatgatggcgtgcagtctataaactgttgcccaccttctgtactttctctcagaataattcacattcttctccagtgtctgttgattgttactttgtggaataagttcttggaaaattccacaagattattgttatcttcttactaccaattctattgaactttctccaccttctctgggccttccccagccagtggtgggaagatgctggctggagtctgacagagcctcttctacactggcctgggcttgctgtgagttggtggaaacctttgctcttgtcccaacacagagcaagtgaaagaggaggtcaaggggctcaggcagcggactagggaagcagaatcgaggaaaaggaaaaatggctgacttattacctcaaaactctagagaatttagttgatcttacagccaagaaggacaaaagccagagagtaatatcctccgcctcatgtctaacccacagaatacatagcaagtaaagagaacatgggcctttataaaaatgtcttaagatacaattttttaattggaggaaatctacagtttaattttctctgggcagcttttcttccttttattatagtaggggaaatcccatgttgatatacttctaaatgaaagatgatgaattgatataatacaataaaaaatctgtaaaattgatgatatacttatcaagaaaaattagctttcattttaacggtttacaaattgagtcaagtcctagtaacaaaatgttaagtctattaacataaccacaagaaatacaggaagacgggcaatctgtgaagcctttcacttacaatctctggcccctcacctgtgctgtgtaggaaaatctttgtgcacaatttgcttccttaattcattttttattcattcaacacattctaataaattatacaaaatcatgttgaaatgtgaatttcagtggtatttataaatgcagtgtgaggagggtttggatgtattctaagacaatagttgtgctttgggaaggaagcagtgttcactgaaaagtgcccccaggaccttttaattggaggaaatatgcttctgtggagttggaaatgggg

SEQ ID NO: 12 - protein, 1140 aa, Homo sapiens
  PEPTIDE (1)..(1140): EGFR Deletion mutant Amino Acids
EITYVQRNYDLSFLKTIQEVAGYVLIALNTVERIPLENLQIIRGNMYYENSYALAVLSNYDANKTGLKELPMRNLQEILHGAVRFSNNPALCNVESIQWRDIVSSDFLSNMSMDFQNHLGSCQKCDPSCPNGSCWGAGEENCQKLTKIICAQQCSGRCRGKSPSDCCHNQCAAGCTGPRESDCLVCRKFRDEATCKDTCPPLMLYNPTTYQMDVNPEGKYSFGATCVKKCPRNYVVTDHGSCVRACGADSYEMEEDGVRKCKKCEGPCRKVCNGIGIGEFKDSLSINATNIKHFKNCTSISGDLHILPVAFRGDSFTHTPPLDPQELDILKTVKEITGFLLIQAWPENRTDLHAFENLEIIRGRTKQHGQFSLAVVSLNITSLGLRSLKEISDGDVIISGNKNLCYANTINWKKLFGTSGQKTKIISNRGENSCKATGQVCHALCSPEGCWGPEPRDCVSCRNVSRGRECVDKCNLLEGEPREFVENSECIQCHPECLPQAMNITCTGRGPDNCIQCAHYIDGPHCVKTCPAGVMGENNTLVWKYADAGHVCHLCHPNCTYGCTGPGLEGCPTNGPKIPSIATGMVGALLLLLVVALGIGLFMRRRHIVRKRTLRRLLQERELVEPLTPSGEAPNQALLRILKETEFKKIKVLGSGAFGTVYKGLWIPEGEKVKIPVAIKTSPKANKEILDEAYVMASVDNPHVCRLLGICLTSTVQLITQLMPFGCLLDYVREHKDNIGSQYLLNWCVQIAKGMNYLEDRRLVHRDLAARNVLVKTPQHVKITDFGLAKLLGAEEKEYHAEGGKVPIKWMALESILHRIYTHQSDVWSYGVTVWELMTFGSKPYDGIPASEISSILEKGERLPQPPICTIDVYMIMVKCWMIDADSRPKFRELIIEFSKMARDPQRYLVIQGDERMHLPSPTDSNFYRALMDEEDMDDVVDADEYLIPQQGFFSSPSTSRTPLLSSLSATSNNSTVACIDRNGLQSCPIKEDSFLQRYSSDPTGALTEDSIDDTFLPVPEYINQSVPKRPAGSVQNPVYHNQPLNPAPSRDPHYQDPHSTAVGNPEYLNTVQPTCVNSTFDSPAHWAQKGSHQISLDNPDYQQDFFPKEAKPNGIFKGSTAENAEYLRVAPQSSEFIGA

SEQ ID NO: 13 - DNA, 23 bp, Artificial Sequence
  EGFR  target site including PAM
tcttaattccttgatagcgacgg

SEQ ID NO: 14 - DNA, 73 bp, Artificial Sequence
  KRAS_F Primer
acactctttccctacacgacgctcttccgatctacattttcattatttttattataaggcctgctgaaaatga

SEQ ID NO: 15 - DNA, 72 bp, Artificial Sequence
  KRAS_R Primer
gtgactggagttcagacgtgtgctcttccgatctttaaaacaagatttacctctattgttggatcatattcg

SEQ ID NO: 16 - DNA, 51 bp, Artificial Sequence
  EGFR_F Primer
cactctttccctacacgacgctcttccgatgggactctggatcccagaagg

SEQ ID NO: 17 - DNA, 52 bp, Artificial Sequence
  EGFR_R Primer
gtgactggagttcagacgtgtgctcttccgatcagctgccagacatgagaaa

SEQ ID NO: 18 - DNA, 33 bp, Artificial Sequence
  Phosphothioate primer_F
acactctttccctacacgacgctcttccgatct

SEQ ID NO: 19 - DNA, 31 bp, Artificial Sequence
  Phosphothioate primer_R
gactggagttcagacgtgtgctcttccgatc